European Patent Application EP 4 119 660 A1, published January 18, 2023. Title: Thermostable phytase variants. Applicant: AB Enzymes. The sequence listing filed with the application follows.

SEQUENCE LISTING (1 sequence)

SEQ ID NO: 1 - protein, 410 aa, Artificial Sequence
  variant
QSEPELKLESVVIVSRHGVRAPTKFTQLMQDVTPDAWPTWPVKLGELTPRGGELIAYLGHYWRQRLVADGLLPKEGCPQSGQVAIIADVDERTRKTGEAFAAGLAPDCAITVHHQADTSSPDPLFNPLKTGVCQLDVANVRRAILERAGGSIADFTRHYQTAFRELERVLNFPQSNLCLKREKQDESCSLTQALPSELKVSADDVSLTGAWSLASMLTEIFLLQQAQGMPEPGWGRITDSHQWNTLLSLHNAVFDLLQRTPEVARSRATPLLDLIKTALTPHPPQKQAYGVTLPTSVLFIAGHDTNLANLGGALELNWTLPGQPDNYPPGGELVFERWRRLSDNSQWIQVSLVFQTLQQMRDKTPLSLNTPPGEVKLTLAGCEERNAQGMCSLAGFTQIVNEARIPACSL